European Patent Application EP 4 276 195 A1, published November 15, 2023. Title: METHODS FOR DETERMINING THE PRESENCE OR RISK OF DEVELOPING MYOTONIC DYSTROPHY TYPE 1 (MD1) OR MYOTONIC DYSTROPHY TYPE 2 (MD2). Applicant: GENARTIS S.R.L. The sequence listing filed with the application follows.

SEQUENCE LISTING (44 sequences)

SEQ ID NO: 1 - RNA, 20 nt, Artificial Sequence
  gRNA1_DMPK
cggacaaccagaacuucgcc

SEQ ID NO: 2 - RNA, 20 nt, Artificial Sequence
  gRNA6_DMPK
ucgagcuugcgucccaggag

SEQ ID NO: 3 - RNA, 20 nt, Artificial Sequence
  gRNA7_DMPK
ggucuucaggaauucuaacg

SEQ ID NO: 4 - RNA, 20 nt, Artificial Sequence
  gRNA8_DMPK
agucccccacguauauggca

SEQ ID NO: 5 - RNA, 20 nt, Artificial Sequence
  gRNA10_DMPK
ucgaucuuugagcugagcgc

SEQ ID NO: 6 - RNA, 20 nt, Artificial Sequence
  gRNA14_DMPK
uucccuggcccaaguuucgg

SEQ ID NO: 7 - RNA, 20 nt, Artificial Sequence
  gRNA15_DMPK
accaaugucgggagaggcca

SEQ ID NO: 8 - RNA, 20 nt, Artificial Sequence
  gRNA16_DMPK
cuggucauggaguauuacgu

SEQ ID NO: 9 - RNA, 20 nt, Artificial Sequence
  gRNA17_DMPK
cguccacuacaaggugagca

SEQ ID NO: 10 - RNA, 20 nt, Artificial Sequence
  gRNA18_DMPK
guguauagacaccuggagga

SEQ ID NO: 11 - RNA, 20 nt, Artificial Sequence
  gRNA1_CNBP
ccaccugauucacugcgaua

SEQ ID NO: 12 - RNA, 20 nt, Artificial Sequence
  gRNA2_CNBP
ggcuucucauuccacgacca

SEQ ID NO: 13 - DNA, 20 bp, Artificial Sequence
  gRNA1_DMPK target sequence
cggacaaccagaacttcgcc

SEQ ID NO: 14 - DNA, 20 bp, Artificial Sequence
  gRNA6_DMPK target sequence
tcgagcttgcgtcccaggag

SEQ ID NO: 15 - DNA, 20 bp, Artificial Sequence
  gRNA7_DMPK target sequence
ggtcttcaggaattctaacg

SEQ ID NO: 16 - DNA, 20 bp, Artificial Sequence
  gRNA8_DMPK target sequence
agtcccccacgtatatggca

SEQ ID NO: 17 - DNA, 20 bp, Artificial Sequence
  gRNA10_DMPK target sequence
tcgatctttgagctgagcgc

SEQ ID NO: 18 - DNA, 20 bp, Artificial Sequence
  gRNA14_DMPK target sequence
ttccctggcccaagtttcgg

SEQ ID NO: 19 - DNA, 20 bp, Artificial Sequence
  gRNA15_DMPK target sequence
accaatgtcgggagaggcca

SEQ ID NO: 20 - DNA, 20 bp, Artificial Sequence
  gRNA16_DMPK target sequence
ctggtcatggagtattacgt

SEQ ID NO: 21 - DNA, 20 bp, Artificial Sequence
  gRNA17_DMPK target sequence
cgtccactacaaggtgagca

SEQ ID NO: 22 - DNA, 20 bp, Artificial Sequence
  gRNA18_DMPK target sequence
gtgtatagacacctggagga

SEQ ID NO: 23 - DNA, 20 bp, Artificial Sequence
  gRNA1_CNBP target sequence
ccacctgattcactgcgata

SEQ ID NO: 24 - DNA, 20 bp, Artificial Sequence
  gRNA2_CNBP target sequence
ggcttctcattccacgacca

SEQ ID NO: 25 - DNA, 42 bp, Artificial Sequence
  CTG repeat
ctgctgctgctgctgctgctgctgctgctgctgctgctgctg

SEQ ID NO: 26 - DNA, 15 bp, Artificial Sequence
  CTG repeat
ctgctgctgctgctg

SEQ ID NO: 27 - DNA, 144 bp, Artificial Sequence
  (TG)20(TCTG)10(CCTG)6(GCTG)1(CCTG)1(TCTG)1(CCTG)7
tgtgtgtgtgtgtgtgtgtgtgtgtgtgtgtgtgtgtgtgtctgtctgtctgtctgtctgtctgtctgtctgtctgtctgcctgcctgcctgcctgcctgcctggctgcctgtctgcctgcctgcctgcctgcctgcctgcctg

SEQ ID NO: 28 - DNA, 20 bp, Artificial Sequence
  gRNA1_DMPK Fw primer
ctgaagtggcagttccagcg

SEQ ID NO: 29 - DNA, 20 bp, Artificial Sequence
  gRNA1_DMPK Rv primer
ctcgcgtagttgactgtggg

SEQ ID NO: 30 - DNA, 20 bp, Artificial Sequence
  gRNA6_DMPK Fw primer
caccgagcgtcgagaagagg

SEQ ID NO: 31 - DNA, 23 bp, Artificial Sequence
  gRNA6_DMPK Rv primer
ggctagaaagtttgcagcaactt

SEQ ID NO: 32 - DNA, 21 bp, Artificial Sequence
  gRNA7_DMPK Fw primer
agggtgtgtcaggtggatgag

SEQ ID NO: 33 - DNA, 20 bp, Artificial Sequence
  gRNA7_DMPK Rv primer
cccagacactccttccctag

SEQ ID NO: 34 - DNA, 20 bp, Artificial Sequence
  gRNA8_DMPK Fw primer
agacgcagggacaggaatgg

SEQ ID NO: 35 - DNA, 21 bp, Artificial Sequence
  gRNA8_DMPK Rv primer
gttccgcttacagctagtacc

SEQ ID NO: 36 - DNA, 22 bp, Artificial Sequence
  gRNA10_DMPK Fw primer
taagtaagggtgtgtgtgttgc

SEQ ID NO: 37 - DNA, 22 bp, Artificial Sequence
  gRNA10_DMPK Rv primer
aacaaatcaggattcccacctg

SEQ ID NO: 38 - DNA, 22 bp, Artificial Sequence
  gRNA1_CNBP Fw Primer
gacaagtctatcacaagggacc

SEQ ID NO: 39 - DNA, 22 bp, Artificial Sequence
  gRNA1_CNBP Rv Primer
taaaagaggtctttgagtggcc

SEQ ID NO: 40 - DNA, 22 bp, Artificial Sequence
  gRNA2_CNBP Fw Primer
caaagatctgactgcagccatg

SEQ ID NO: 41 - DNA, 22 bp, Artificial Sequence
  gRNA2_CNBP Rv Primer
gacaaaatacctctatccgagg

SEQ ID NO: 42 - DNA, 20 bp, Artificial Sequence
  PRL Fw primer
agggaaacgaatgcctgatt

SEQ ID NO: 43 - DNA, 20 bp, Artificial Sequence
  PRL Rv primer
gcaggaaacacacttcacca

SEQ ID NO: 44 - DNA, 10 bp, Artificial Sequence
  (TG)v(TCTG)w(CCTG)x motif
  repeat_region 2: /rpt_unit_seq="TG repeat"
  repeat_region 6: /rpt_unit_seq="TCTG repeat"
  repeat_region 10: /rpt_unit_seq="CCTG repeat"
tgtctgcctg